European Patent Application EP 4 242 315 A1, published September 13, 2023. Title: Mutant ATP-dependent protease and method for producing L-amino acid using the same. Applicant: CJ CheilJedang Corporation. The sequence listing filed with the application follows.

SEQUENCE LISTING (26 sequences)

SEQ ID NO: 1 - protein, 922 aa, Artificial Sequence
  ClpC variant ORF AA
MFERFTDRARRVIVLAQEEARMLNHNYIGTEHILLGLIHEGEGVAAKALESMGISLDAVRQEVEEIIGQGSQPTTGHIPFTPRAKKVLELSLREGLQMGHKYIGTEFLLLGLIREGEGVAAQVLVKLGADLPRVRQQVIQLLSGYEGGQGGSPEGGQGAPTGGDAVGAGAAPGGRPSSGGPGERSTSLVLDQFGRNLTQAAKDGKLDPVVGRDKEIERIMQVLSRRTKNNPVLIGEPGVGKTAVVEGLALDIVNGKVPETLKDKQVYSLDLGSLVAGSRYRGDFEERLKKVLKEINQRGDIILFIDEIHTLVGAGAAEGAIDAASLLKPKLARGELQTIGATTLDEYRKHIEKDAALERRFQPVQVPEPSVDLTVEILKGLRDRYEAHHRVSITDGALTAAAQLADRYINDRFLPDKAVDLIDEAGARMRMTAPSSLREVDERIADVRREKEAAIDAQDFEKAAGLRDKERKLGEERSEKEKQWRSGDLEDIAEVGEEQIAEVLANWTGIPVFKLTEAESSRLLNMEEELHKRIIGQDEAVKAVSRAIRRTRAGLKDPKRPSGSFIFAGPSGVGKTELSKALAGFLFGDDDSLIQIDMGEFHDRFTASRLFGAPPGYVGYEEGGQLTEKVRRKPFSVVLFDEIEKAHKEIYNTLLQVLEDGRLTDGQGRIVDFKNTVLIFTSNLGTSDISKAVGLGFSGSSETDSDAQYDRMKNKVHDELKKHFRPEFLNRIDEIVVFHQLTKDQIVQMVDLLIGRVSNALAEKDMSIELTEKAKDLLASRGFDPVLGARPLRRTIQREIEDQMSEKILFGEIGAGEIVTVDVEGWDGESKDTDRAKFTFTPRPKPMPEGKFSEISVQAAEAIQDVDSAADGDVPETDSLSDIDLETLEKFEEDVENGTDIDQVSGDYYGTDDQGGTAPSKE

SEQ ID NO: 2 - DNA, 2769 bp, Artificial Sequence
  clpC variant ORF NT
atgttcgagaggtttaccgatcgtgcacgccgcgtgattgtgctcgcgcaggaagaggcgcgcatgctcaaccacaattacatcggcacggagcacattctcctcggcctcattcacgagggcgagggcgttgcagccaaggctttggaatccatgggaatttccctggacgccgtccgccaggaagtcgaagagattatcggccagggctcccagcccaccaccggccacattccttttactccacgtgccaagaaggtcctggagctcagcctccgcgagggactacagatgggacacaagtacatcggtactgagttcctgcttctcggtttgatccgtgagggcgagggcgttgctgcccaggtcctggtcaagcttggtgctgatctgccacgcgtgcgtcagcaagttattcagcttctctccggctacgaaggtggccagggcggatccccagagggcggtcagggcgcccctactggcggtgacgctgttggtgcaggagctgctcctggcggtcgtccatcttcgggcggcccaggcgagcgttctacctctttggttcttgaccagttcggccgcaacctcacccaggccgcaaaggacggcaagctggacccagttgttggtcgtgataaggaaatcgagcgcatcatgcaggtgctctcccgtcgtaccaagaacaacccagttcttattggtgagccaggtgttggtaagaccgcagttgttgaaggtcttgcactagacattgttaacggcaaggttccagagaccctcaaggacaagcaggtttactcccttgacttaggttcactggttgcaggttcccgttaccgcggtgacttcgaagagcgcctgaagaaggtcctcaaggagattaaccagcgcggcgacatcatcctgtttatcgatgagatccacaccctcgtgggtgcaggtgcagcagaaggcgcaatcgacgccgcctccctgcttaagccaaagcttgcccgcggtgaactgcagaccattggtgcaaccaccttggacgagtaccgtaagcacattgaaaaggacgcagctcttgagcgtcgtttccagccagtgcaggttccagagccttcggttgatctcaccgttgagatcttgaagggtctgcgcgaccgctacgaagctcaccaccgcgtatccatcaccgatggtgctcttaccgcagcagctcagcttgctgatcgctacattaacgaccgcttcttgccagataaggccgttgacctcatcgatgaggctggcgcccgcatgcgcatgaccgcaccgtcctccctccgcgaggttgatgagcgcatcgctgatgttcgccgtgagaaggaagcagcgatcgatgctcaggactttgagaaggcagcaggtcttcgcgataaggagcgcaagctcggcgaagagcgttcagagaaggaaaagcagtggcgctccggcgacctcgaggacattgctgaggttggcgaagagcagatcgcagaagtactggccaactggactggtattcctgtcttcaagctcaccgaagctgagtcttcccgcctgctcaacatggaagaagagttgcacaagcgcatcatcggacaggatgaagctgtcaaggctgtctcccgtgcgatccgtcgtacccgtgcaggtctgaaggatcctaagcgtccttccggctccttcatcttcgctggtccatccggtgttggtaagaccgagctgtccaaggcacttgctggattcctcttcggtgacgatgattccctcatccaaatcgacatgggtgaattccacgaccgcttcaccgcgtcccgactcttcggtgcccctccgggatacgttggctacgaagaaggtggccagctgaccgagaaggttcgccgtaagccattctccgttgtgcttttcgacgagatcgagaaggcccacaaggagatctacaacaccttgctgcaggtgttggaagatggtcgccttaccgatggtcagggtcgcattgtggacttcaagaacaccgtcctgatcttcacctccaacctgggcacctctgacatctccaaggctgttggcctgggcttctccggatcctctgagactgacagcgatgctcagtacgaccgcatgaagaacaaggtccacgacgagctgaagaagcacttccgccctgagttcctgaaccgtattgatgagatcgtggtcttccaccagctcaccaaggatcagatcgttcagatggtcgaccttcttattggccgcgtgtccaacgcactggctgagaaggacatgagcatcgaactgactgagaaggctaaggatctccttgccagccgcggcttcgatccagttctgggtgcacgaccattgcgtcgcaccattcagcgcgaaatcgaagaccagatgtccgagaagatcctcttcggagaaatcggtgctggcgagatcgtcaccgtcgacgtcgaaggctgggacggcgagtccaaggacaccgaccgtgcgaagttcaccttcacaccacgtccaaagccaatgccagaaggtaagttctctgagatctccgtacaggctgcagaagcaatccaagatgtagattccgcagctgacggcgatgtcccagaaaccgattcactttccgacattgaccttgaaacccttgagaagttcgaggaagatgtagaaaacggcaccgacattgatcaggtatccggtgactactacggcaccgatgatcagggaggcactgctccaagcaaggagtag

SEQ ID NO: 3 - protein, 3 aa, Artificial Sequence
  431~433  AA
IKR

SEQ ID NO: 4 - DNA, 9 bp, Artificial Sequence
  1,291~1,299 NT
atcaagcgc

SEQ ID NO: 5 - protein, 925 aa, Unknown
  ClpC ORF WT AA
MFERFTDRARRVIVLAQEEARMLNHNYIGTEHILLGLIHEGEGVAAKALESMGISLDAVRQEVEEIIGQGSQPTTGHIPFTPRAKKVLELSLREGLQMGHKYIGTEFLLLGLIREGEGVAAQVLVKLGADLPRVRQQVIQLLSGYEGGQGGSPEGGQGAPTGGDAVGAGAAPGGRPSSGGPGERSTSLVLDQFGRNLTQAAKDGKLDPVVGRDKEIERIMQVLSRRTKNNPVLIGEPGVGKTAVVEGLALDIVNGKVPETLKDKQVYSLDLGSLVAGSRYRGDFEERLKKVLKEINQRGDIILFIDEIHTLVGAGAAEGAIDAASLLKPKLARGELQTIGATTLDEYRKHIEKDAALERRFQPVQVPEPSVDLTVEILKGLRDRYEAHHRVSITDGALTAAAQLADRYINDRFLPDKAVDLIDEAGARMRIKRMTAPSSLREVDERIADVRREKEAAIDAQDFEKAAGLRDKERKLGEERSEKEKQWRSGDLEDIAEVGEEQIAEVLANWTGIPVFKLTEAESSRLLNMEEELHKRIIGQDEAVKAVSRAIRRTRAGLKDPKRPSGSFIFAGPSGVGKTELSKALAGFLFGDDDSLIQIDMGEFHDRFTASRLFGAPPGYVGYEEGGQLTEKVRRKPFSVVLFDEIEKAHKEIYNTLLQVLEDGRLTDGQGRIVDFKNTVLIFTSNLGTSDISKAVGLGFSGSSETDSDAQYDRMKNKVHDELKKHFRPEFLNRIDEIVVFHQLTKDQIVQMVDLLIGRVSNALAEKDMSIELTEKAKDLLASRGFDPVLGARPLRRTIQREIEDQMSEKILFGEIGAGEIVTVDVEGWDGESKDTDRAKFTFTPRPKPMPEGKFSEISVQAAEAIQDVDSAADGDVPETDSLSDIDLETLEKFEEDVENGTDIDQVSGDYYGTDDQGGTAPSKE

SEQ ID NO: 6 - DNA, 2778 bp, Unknown
  clpC ORF WT NT
atgttcgagaggtttaccgatcgtgcacgccgcgtgattgtgctcgcgcaggaagaggcgcgcatgctcaaccacaattacatcggcacggagcacattctcctcggcctcattcacgagggcgagggcgttgcagccaaggctttggaatccatgggaatttccctggacgccgtccgccaggaagtcgaagagattatcggccagggctcccagcccaccaccggccacattccttttactccacgtgccaagaaggtcctggagctcagcctccgcgagggactacagatgggacacaagtacatcggtactgagttcctgcttctcggtttgatccgtgagggcgagggcgttgctgcccaggtcctggtcaagcttggtgctgatctgccacgcgtgcgtcagcaagttattcagcttctctccggctacgaaggtggccagggcggatccccagagggcggtcagggcgcccctactggcggtgacgctgttggtgcaggagctgctcctggcggtcgtccatcttcgggcggcccaggcgagcgttctacctctttggttcttgaccagttcggccgcaacctcacccaggccgcaaaggacggcaagctggacccagttgttggtcgtgataaggaaatcgagcgcatcatgcaggtgctctcccgtcgtaccaagaacaacccagttcttattggtgagccaggtgttggtaagaccgcagttgttgaaggtcttgcactagacattgttaacggcaaggttccagagaccctcaaggacaagcaggtttactcccttgacttaggttcactggttgcaggttcccgttaccgcggtgacttcgaagagcgcctgaagaaggtcctcaaggagattaaccagcgcggcgacatcatcctgtttatcgatgagatccacaccctcgtgggtgcaggtgcagcagaaggcgcaatcgacgccgcctccctgcttaagccaaagcttgcccgcggtgaactgcagaccattggtgcaaccaccttggacgagtaccgtaagcacattgaaaaggacgcagctcttgagcgtcgtttccagccagtgcaggttccagagccttcggttgatctcaccgttgagatcttgaagggtctgcgcgaccgctacgaagctcaccaccgcgtatccatcaccgatggtgctcttaccgcagcagctcagcttgctgatcgctacattaacgaccgcttcttgccagataaggccgttgacctcatcgatgaggctggcgcccgcatgcgcatcaagcgcatgaccgcaccgtcctccctccgcgaggttgatgagcgcatcgctgatgttcgccgtgagaaggaagcagcgatcgatgctcaggactttgagaaggcagcaggtcttcgcgataaggagcgcaagctcggcgaagagcgttcagagaaggaaaagcagtggcgctccggcgacctcgaggacattgctgaggttggcgaagagcagatcgcagaagtactggccaactggactggtattcctgtcttcaagctcaccgaagctgagtcttcccgcctgctcaacatggaagaagagttgcacaagcgcatcatcggacaggatgaagctgtcaaggctgtctcccgtgcgatccgtcgtacccgtgcaggtctgaaggatcctaagcgtccttccggctccttcatcttcgctggtccatccggtgttggtaagaccgagctgtccaaggcacttgctggattcctcttcggtgacgatgattccctcatccaaatcgacatgggtgaattccacgaccgcttcaccgcgtcccgactcttcggtgcccctccgggatacgttggctacgaagaaggtggccagctgaccgagaaggttcgccgtaagccattctccgttgtgcttttcgacgagatcgagaaggcccacaaggagatctacaacaccttgctgcaggtgttggaagatggtcgccttaccgatggtcagggtcgcattgtggacttcaagaacaccgtcctgatcttcacctccaacctgggcacctctgacatctccaaggctgttggcctgggcttctccggatcctctgagactgacagcgatgctcagtacgaccgcatgaagaacaaggtccacgacgagctgaagaagcacttccgccctgagttcctgaaccgtattgatgagatcgtggtcttccaccagctcaccaaggatcagatcgttcagatggtcgaccttcttattggccgcgtgtccaacgcactggctgagaaggacatgagcatcgaactgactgagaaggctaaggatctccttgccagccgcggcttcgatccagttctgggtgcacgaccattgcgtcgcaccattcagcgcgaaatcgaagaccagatgtccgagaagatcctcttcggagaaatcggtgctggcgagatcgtcaccgtcgacgtcgaaggctgggacggcgagtccaaggacaccgaccgtgcgaagttcaccttcacaccacgtccaaagccaatgccagaaggtaagttctctgagatctccgtacaggctgcagaagcaatccaagatgtagattccgcagctgacggcgatgtcccagaaaccgattcactttccgacattgaccttgaaacccttgagaagttcgaggaagatgtagaaaacggcaccgacattgatcaggtatccggtgactactacggcaccgatgatcagggaggcactgctccaagcaaggagtag

SEQ ID NO: 7 - DNA, 35 bp, Artificial Sequence
  P1
ctattctagatccagagaccctcaaggacaagcag

SEQ ID NO: 8 - DNA, 30 bp, Artificial Sequence
  P2
ggacggtgcggtcatgcgcatgcgggcgcc

SEQ ID NO: 9 - DNA, 30 bp, Artificial Sequence
  P3
ggcgcccgcatgcgcatgaccgcaccgtcc

SEQ ID NO: 10 - DNA, 34 bp, Artificial Sequence
  P4
ctattctagatcgatttggatgagggaatcatcg

SEQ ID NO: 11 - DNA, 32 bp, Artificial Sequence
  P5
aatttctagaggcagaccctattctatgaagg

SEQ ID NO: 12 - DNA, 30 bp, Artificial Sequence
  P6
agtgtttcggtctttacagacacgagggac

SEQ ID NO: 13 - DNA, 30 bp, Artificial Sequence
  P7
gtccctcgtgtctgtaaagaccgaaacact

SEQ ID NO: 14 - DNA, 32 bp, Artificial Sequence
  P8
aatttctagacgtgggagtgtcactcgcttgg

SEQ ID NO: 15 - DNA, 29 bp, Artificial Sequence
  P9
tcctctagagctgcgcagtgttgaatacg

SEQ ID NO: 16 - DNA, 30 bp, Artificial Sequence
  P10
tggaaatcttttcgatgttcacgttgacat

SEQ ID NO: 17 - DNA, 30 bp, Artificial Sequence
  P11
acatcgaaaagatttccacctctgagattc

SEQ ID NO: 18 - DNA, 29 bp, Artificial Sequence
  P12
gactctagagttcacctcagagacgatta

SEQ ID NO: 19 - DNA, 29 bp, Artificial Sequence
  P13
tcctctagactggtcgcctgatgttctac

SEQ ID NO: 20 - DNA, 23 bp, Artificial Sequence
  P14
cacgatcagatgtgcatcatcat

SEQ ID NO: 21 - DNA, 23 bp, Artificial Sequence
  P15
atgatgatgcacatctgatcgtg

SEQ ID NO: 22 - DNA, 29 bp, Artificial Sequence
  P16
gactctagattagtccctttcgaggcgga

SEQ ID NO: 23 - DNA, 28 bp, Artificial Sequence
  P17
acggatcccagactccaaagcaaaagcg

SEQ ID NO: 24 - DNA, 30 bp, Artificial Sequence
  P18
acaccacggcagaaccaggtgcaaaggaca

SEQ ID NO: 25 - DNA, 30 bp, Artificial Sequence
  P19
ctggttctgccgtggtgtgcatcatctctg

SEQ ID NO: 26 - DNA, 28 bp, Artificial Sequence
  P20
acggatccaaccaaacttgctcacactc